European Patent Specification EP 4 210 761 B1, published August 20, 2025. Title: SEMICARBAZONE-BASED SAPONIN CONJUGATE. Applicant: Sapreme Technologies B.V. The sequence listing filed with the application follows.

SEQUENCE LISTING (22 sequences)

SEQ ID NO: 1 - DNA, 16 bp, Artificial Sequence
  Antisense BNA (HSP27) oligo nucleic acid sequence
ggcacagccagtggcg

SEQ ID NO: 2 - DNA, 20 bp, Artificial Sequence
  HSP27 primer forward sequence
gcagtccaacgagatcacca

SEQ ID NO: 3 - DNA, 20 bp, Artificial Sequence
  HSP27 primer reverse sequence
taaggctttacttggcggca

SEQ ID NO: 4 - DNA, 20 bp, Artificial Sequence
  HBMS primer forward sequence
cacccacacacagcctactt

SEQ ID NO: 5 - DNA, 20 bp, Artificial Sequence
  HBMS primer reverse sequence
gtacccacgcgaatcactct

SEQ ID NO: 6 - DNA, 22 bp, Artificial Sequence
  GUSB primer forward sequence
gaaaatacgtggttggagagct

SEQ ID NO: 7 - DNA, 22 bp, Artificial Sequence
  GUSB primer reverse sequence
ccgagtgaagatccccttttta

SEQ ID NO: 8 - DNA, 20 bp, Artificial Sequence
  APOB BNA oligo
gcctcagtctgcttcgcacc

SEQ ID NO: 9 - DNA, 20 bp, Artificial Sequence
  APOB scrambled BNA oligo
ggcctctctacaccgctcgt

SEQ ID NO: 10 - DNA, 20 bp, Artificial Sequence
  HSP27 primer forward sequence
gcagtccaacgagatcacca

SEQ ID NO: 11 - DNA, 20 bp, Artificial Sequence
  HSP27 primer reverse sequence
taaggctttacttggcggca

SEQ ID NO: 12 - DNA, 20 bp, Artificial Sequence
  ApoB primer forward sequence
agggtccgggaatctgatga

SEQ ID NO: 13 - DNA, 21 bp, Artificial Sequence
  ApoB primer reverse sequence
tgggcacgttgtctttcagag

SEQ ID NO: 14 - DNA, 13 bp, Artificial Sequence
  ApoB#02
gcattggtattca

SEQ ID NO: 15 - DNA, 24 bp, Artificial Sequence
  ApoB#02 forward primer
gctaacactaagaaccagaagatc

SEQ ID NO: 16 - DNA, 20 bp, Artificial Sequence
  ApoB#02 reverse primer
tgtccgtctaaggatcctgc

SEQ ID NO: 17 - DNA, 18 bp, Artificial Sequence
  Mm PPIA forward primer
gcggcaggtccatctacg

SEQ ID NO: 18 - DNA, 19 bp, Artificial Sequence
  Mm PPIA reverse primer
gccatccagccattcagtc

SEQ ID NO: 19 - DNA, 20 bp, Artificial Sequence
  Mm SDHA forward primer
gaggaagcacaccctctcat

SEQ ID NO: 20 - DNA, 20 bp, Artificial Sequence
  Mm SDHA reverse primer
ggagcggatagcaggaggta

SEQ ID NO: 21 - DNA, 20 bp, Artificial Sequence
  Mm RPS17 forward primer
gtgcgaggagatcgccatta

SEQ ID NO: 22 - DNA, 20 bp, Artificial Sequence
  Mm RPS17 reverse primer
atccgcttcatcagatgcgt